European Patent Application EP 4 183 868 A1, published May 24, 2023. Title: Off-the-shelf stem cell and immune cell, and a pharmaceutical composition. Applicant: KANGSTEM BIOTECH CO., LTD. The sequence listing filed with the application follows.

SEQUENCE LISTING (13 sequences)

SEQ ID NO: 1 - RNA, 20 nt, Artificial Sequence
  B2M sgRNA
actcacgctggatagcctcc

SEQ ID NO: 2 - RNA, 20 nt, Artificial Sequence
  CIITA sgRNA
gatattggcataagcctccc

SEQ ID NO: 3 - RNA, 20 nt, Artificial Sequence
  PDCD1 sgRNA
atgtggaagtcacgcccgtt

SEQ ID NO: 4 - RNA, 20 nt, Artificial Sequence
  CTLA4 sgRNA
gtgcggcaacctacatgatg

SEQ ID NO: 5 - RNA, 20 nt, Artificial Sequence
  TRA sgRNA
ctctcagctggtacacggca

SEQ ID NO: 6 - RNA, 243 nt, Homo sapiens
atgggcagagcaatggtggccaggctcgggctggggctgctgctgctggcactgctcctacccacgcagatttattccagtgaaacaacaactggaacttcaagtaactcctcccagagtacttccaactctgggttggccccaaatccaactaatgccaccaccaaggcggctggtggtgccctgcagtcaacagccagtctcttcgtggtctcactctctcttctgcatctctactcttaa

SEQ ID NO: 7 - DNA, 10843 bp, Artificial Sequence
  CD19 CAR whole vector
tggacggcgacgtaaacggccacaagcgataccgtcgacctcgagggaattaattcgagctcggtacctttaagaccaatgacttacaaggcagctgtagatcttagccactttttaaaagaaaaggggggactggaagggctaattcactcccaacgaagacaagatctgctttttgcttgtactgggtctctctggttagaccagatctgagcctgggagctctctggctaactagggaacccactgcttaagcctcaataaagcttgccttgagtgcttcaagtagtgtgtgcccgtctgttgtgtgactctggtaactagagatccctcagacccttttagtcagtgtggaaaatctctagcagcatctagaattaattccgtgtattctatagtgtcacctaaatcgtatgtgtatgatacataaggttatgtattaattgtagccgcgttctaacgacaatatgtacaagcctaattgtgtagcatctggcttactgaagcagaccctatcatctctctcgtaaactgccgtcagagtcggtttggttggacgaaccttctgagtttctggtaacgccgtcccgcacccggaaatggtcagcgaaccaatcagcagggtcatcgctagccagatcctctacgccggacgcatcgtggccggcatcaccggcgccacaggtgcggttgctggcgcctatatcgccgacatcaccgatggggaagatcgggctcgccacttcgggctcatgagcgcttgtttcggcgtgggtatggtggcaggccccgtggccgggggactgttgggcgccatctccttgcatgcaccattccttgcggcggcggtgctcaacggcctcaacctactactgggctgcttcctaatgcaggagtcgcataagggagagcgtcgaatggtgcactctcagtacaatctagctctgatgccgcatagttaagccagccccgacacccgccaacacccgctgacgcgccctgacgggcttgtctgctcccggcatccgcttacagacaagctgtgaccgtctccgggagctgcatgtgtcagaggttttcaccgtcatcaccgaaacgcgcgagacgaaagggcctcgtgatacgcctatttttataggttaatgtcatgataataatggtttcttagacgtcaggtggcacttttcggggaaatgtgcgcggaacccctatttgtttatttttctaaatacattcaaatatgtatccgctcatgagacaataaccctgataaatgcttcaataatattgaaaaaggaagagtatgagtattcaacatttccgtgtcgcccttattcccttttttgcggcattttgccttcctgtttttgctcacccagaaacgctggtgaaagtaaaagatgctgaagatcagttgggtgcacgagtgggttacatcgaactggatctcaacagcggtaagatccttgagagttttcgccccgaagaacgttttccaatgatgagcacttttaaagttctgctatgtggcgcggtattatcccgtattgacgccgggcaagagcaactcggtcgccgcatacactattctcagaatgacttggttgagtactcaccagtcacagaaaagcatcttacggatggcatgacagtaagagaattatgcagtgctgccataaccatgagtgataacactgcggccaacttacttctgacaacgatcggaggaccgaaggagctaaccgcttttttgcacaacatgggggatcatgtaactcgccttgatcgttgggaaccggagctgaatgaagccataccaaacgacgagcgtgacaccacgatgcctgtagcaatggcaacaacgttgcgcaaactattaactggcgaactacttactctagcttcccggcaacaattaatagactggatggaggcggataaagttgcaggaccacttctgcgctcggcccttccggctggctggtttattgctgataaatctggagccggtgagcgtgggtctcgcggtatcattgcagcactggggccagatggtaagccctcccgtatcgtagttatctacacgacggggagtcaggcaactatggatgaacgaaatagacagatcgctgagataggtgcctcactgattaagcattggtaactgtcagaccaagtttactcatatatactttagattgatttaaaacttcatttttaatttaaaaggatctaggtgaagatcctttttgataatctcatgaccaaaatcccttaacgtgagttttcgttccactgagcgtcagaccccgtagaaaagatcaaaggatcttcttgagatcctttttttctgcgcgtaatctgctgcttgcaaacaaaaaaaccaccgctaccagcggtggtttgtttgccggatcaagagctaccaactctttttccgaaggtaactggcttcagcagagcgcagataccaaatactgtccttctagtgtagccgtagttaggccaccacttcaagaactctgtagcaccgcctacatacctcgctctgctaatcctgttaccagtggctgctgccagtggcgataagtcgtgtcttaccgggttggactcaagacgatagttaccggataaggcgcagcggtcgggctgaacggggggttcgtgcacacagcccagcttggagcgaacgacctacaccgaactgagatacctacagcgtgagctatgagaaagcgccacgcttcccgaagggagaaaggcggacaggtatccggtaagcggcagggtcggaacaggagagcgcacgagggagcttccagggggaaacgcctggtatctttatagtcctgtcgggtttcgccacctctgacttgagcgtcgatttttgtgatgctcgtcaggggggcggagcctatggaaaaacgccagcaacgcggcctttttacggttcctggccttttgctggccttttgctcacatgttctttcctgcgttatcccctgattctgtggataaccgtattaccgcctttgagtgagctgataccgctcgccgcagccgaacgaccgagcgcagcgagtcagtgagcgaggaagcggaagagcgcccaatacgcaaaccgcctctccccgcgcgttggccgattcattaatgcagctgtggaatgtgtgtcagttagggtgtggaaagtccccaggctccccagcaggcagaagtatgcaaagcatgcatctcaattagtcagcaaccaggtgtggaaagtccccaggctccccagcaggcagaagtatgcaaagcatgcatctcaattagtcagcaaccatagtcccgcccctaactccgcccatcccgcccctaactccgcccagttccgcccattctccgccccatggctgactaattttttttatttatgcagaggccgaggccgcctcggcctctgagctattccagaagtagtgaggaggcttttttggaggcctaggcttttgcaaaaagcttggacacaagacaggcttgcgagatatgtttgagaataccactttatcccgcgtcagggagaggcagtgcgtaaaaagacgcggactcatgtgaaatactggtttttagtgcgccagatctctataatctcgcgcaacctattttcccctcgaacactttttaagccgtagataaacaggctgggacacttcacatgagcgaaaaatacatcgtcacctgggacatgttgcagatccatgcacgtaaactcgcaagccgactgatgccttctgaacaatggaaaggcattattgccgtaagccgtggcggtctgtaccgggtgcgttactggcgcgtgaactgggtattcgtcatgtcgataccgtttgtatttccagctacgatcacgacaaccagcgcgagcttaaagtgctgaaacgcgcagaaggcgatggcgaaggcttcatcgttattgatgacctggtggataccggtggtactgcggttgcgattcgtgaaatgtatccaaaagcgcactttgtcaccatcttcgcaaaaccggctggtcgtccgctggttgatgactatgttgttgatatcccgcaagatacctggattgaacagccgtgggatatgggcgtcgtattcgtcccgccaatctccggtcgctaatcttttcaacgcctggcactgccgggcgttgttctttttaacttcaggcgggttacaatagtttccagtaagtattctggaggctgcatccatgacacaggcaaacctgagcgaaaccctgttcaaaccccgctttaaacatcctgaaacctcgacgctagtccgccgctttaatcacggcgcacaaccgcctgtgcagtcggcccttgatggtaaaaccatccctcactggtatcgcatgattaaccgtctgatgtggatctggcgcggcattgacccacgcgaaatcctcgacgtccaggcacgtattgtgatgagcgatgccgaacgtaccgacgatgatttatacgatacggtgattggctaccgtggcggcaactggatttatgagtgggccccggatctttgtgaaggaaccttacttctgtggtgtgacataattggacaaactacctacagagatttaaagctctaaggtaaatataaaatttttaagtgtataatgtgttaaactactgattctaattgtttgtgtattttagattccaacctatggaactgatgaatgggagcagtggtggaatgcctttaatgaggaaaacctgttttgctcagaagaaatgccatctagtgatgatgaggctactgctgactctcaacattctactcctccaaaaaagaagagaaaggtagaagaccccaaggactttccttcagaattgctaagttttttgagtcatgctgtgtttagtaatagaactcttgcttgctttgctatttacaccacaaaggaaaaagctgcactgctatacaagaaaattatggaaaaatattctgtaacctttataagtaggcataacagttataatcataacatactgttttttcttactccacacaggcatagagtgtctgctattaataactatgctcaaaaattgtgtacctttagctttttaatttgtaaaggggttaataaggaatatttgatgtatagtgccttgactagagatcataatcagccataccacatttgtagaggttttacttgctttaaaaaacctcccacacctccccctgaacctgaaacataaaatgaatgcaattgttgttgttaacttgtttattgcagcttataatggttacaaataaagcaatagcatcacaaatttcacaaataaagcatttttttcactgcattctagttgtggtttgtccaaactcatcaatgtatcttatcatgtctggatcaactggataactcaagctaaccaaaatcatcccaaacttcccaccccataccctattaccactgccaattacctagtggtttcatttactctaaacctgtgattcctctgaattattttcattttaaagaaattgtatttgttaaatatgtactacaaacttagtagttggaagggctaattcactcccaaagaagacaagatatccttgatctgtggatctaccacacacaaggctacttccctgattagcagaactacacaccagggccaggggtcagatatccactgacctttggatggtgctacaagctagtaccagttgagccagataaggtagaagaggccaataaaggagagaacaccagcttgttacaccctgtgagcctgcatgggatggatgacccggagagagaagtgttagagtggaggtttgacagccgcctagcatttcatcacgtggcccgagagctgcatccggagtacttcaagaactgctgatatcgagcttgctacaagggactttccgctggggactttccagggaggcgtggcctgggcgggactggggagtggcgagccctcagatcctgcatataagcagctgctttttgcctgtactgggtctctctggttagaccagatctgagcctgggagctctctggctaactagggaacccactgcttaagcctcaataaagcttgccttgagtgcttcaagtagtgtgtgcccgtctgttgtgtgactctggtaactagagatccctcagacccttttagtcagtgtggaaaatctctagcagtggcgcccgaacagggacttgaaagcgaaagggaaaccagaggagctctctcgacgcaggactcggcttgctgaagcgcgcacggcaagaggcgaggggcggcgactggtgagtacgccaaaaattttgactagcggaggctagaaggagagagatgggtgcgagagcgtcagtattaagcgggggagaattagatcgcgatgggaaaaaattcggttaaggccagggggaaagaaaaaatataaattaaaacatatagtatgggcaagcagggagctagaacgattcgcagttaatcctggcctgttagaaacatcagaaggctgtagacaaatactgggacagctacaaccatcccttcagacaggatcagaagaacttagatcattatataatacagtagcaaccctctattgtgtgcatcaaaggatagagataaaagacaccaaggaagctttagacaagatagaggaagagcaaaacaaaagtaagaccaccgcacagcaagcggccggtgatcttcagacctggacgatatatatgagggacaattggagaagtgaattatataaatataaagtagtaaaaattgaaccattaggagtagcacccaccaaggcaaagagaagagtggtgcagagagaaaaaagagcagtgggaataggagctttgttccttgggttcttgggagcagcaggaagcactatgggcgcagcgtcaatgacgctgacggtacaggccagacaattattgtctggtatagtgcagcagcagaacaatttgctgagggctattgaggcgcaacagcatctgttgcaactcacagtctggggcatcaagcagctccaggcaagaatcctggctgtggaaagatacctaaaggatcaacagctcctggggatttggggttgctctggaaaactcatttgcaccactgctgtgccttggaatgctagttggagtaataaatctctggaacagatttggaatcacacgacctggatggagtgggacagagaaattaacaattacacaagcttaatacactccttaattgaagaatcgcaaaaccagcaagaaaagaatgaacaagaattattggaattagataaatgggcaagtttgtggaattggtttaacataacaaattggctgtggtatataaaattattcataatgatagtaggaggcttggtaggtttaagaatagtttttgctgtactttctatagtgaatagagttaggcagggatattcaccattatcgtttcagacccacctcccaaccccgaggggacccgacaggcccgaaggaatagaagaagaaggtggagagagagacagagacagatccattcgattagtgaacggatctcgacggtatcgccaaatggcagtattcatccacaattttaaaagaaaaggggggattggggggtacagtgcaggggaaagaatagtagacataatagcaacagacatacaaactaaagaattacaaaaacaaattacaaaaattcaaaattttcgggtttattacagggacagcagagatccagtttggatcgataagcttgatatcgaattcctgcagccccgataaaataaaagattttatttagtctccagaaaaaggggggaatgaaagaccccacctgtaggtttggcaagctagctgcagtaacgccattttgcaaggcatggaaaaataccaaaccaagaatagagaagttcagatcaagggcgggtacatgaaaatagctaacgttgggccaaacaggatatctgcggtgagcagtttcggccccggcccggggccaagaacagatggtcaccgcagtttcggccccggcccgaggccaagaacagatggtccccagatatggcccaaccctcagcagtttcttaagacccatcagatgtttccaggctcccccaaggacctgaaatgaccctgcgccttatttgaattaaccaatcagcctgcttctcgcttctgttcgcgcgcttctgcttcccgagctctataaaagagctcacaacccctcactcggcgcgccagtcctccgacagactgagtcgcccgggggggatctggagctctcgagaattctcacgcgtgccaccatggccttaccagtgaccgccttgctcctgccgctggccttgctgctccacgccgccaggccggacatccagatgacacagactacatcctccctgtctgcctctctgggagacagagtcaccatcagttgcagggcaagtcaggacattagtaaatatttaaattggtatcagcagaaaccagatggaactgttaaactcctgatctaccatacatcaagattacactcaggagtcccatcaaggttcagtggcagtgggtctggaacagattattctctcaccattagcaacctggagcaagaagatattgccacttacttttgccaacagggtaatacgcttccgtacacgttcggaggggggaccaagctggagatcacaggtggcggtggctcgggcggtggtgggtcgggtggcggcggatctgaggtgaaactgcaggagtcaggacctggcctggtggcgccctcacagagcctgtccgtcacatgcactgtctcaggggtctcattacccgactatggtgtaagctggattcgccagcctccacgaaagggtctggagtggctgggagtaatatggggtagtgaaaccacatactataattcagctctcaaatccagactgaccatcatcaaggacaactccaagagccaagttttcttaaaaatgaacagtctgcaaactgatgacacagccatttactactgtgccaaacattattactacggtggtagctatgctatggactactggggccaaggaacctcagtcaccgtctcctcaaccacgacgccagcgccgcgaccaccaacaccggcgcccaccatcgcgtcgcagcccctgtccctgcgcccagaggcgtgccggccagcggcggggggcgcagtgcacacgagggggctggacttcgcctgtgatatctacatctgggcgcccttggccgggacttgtggggtccttctcctgtcactggttatcaccctttactgcagacgactcaagatccaggtccgaaaggcagctatagccagccgtgagaaagcagatgctgtctacacgggcctgaacacccggagccaggagacatatgagactctgaagcatgagaaaccaccccagggatccggaagtatggtgagcaagggcgaggagctgttcaccggggtggtgcccatcctggtcgagctggacggcgacgtaaacggccacaagttcagcgtgtccggcgagggcgagggcgatgccacctacggcaagctgaccctgaagttcatctgcaccaccggcaagctgcccgtgccctggcccaccctcgtgaccaccctgacctacggcgtgcagtgcttcagccgctaccccgaccacatgaagcagcacgacttcttcaagtccgccatgcccgaaggctacgtccaggagcgcaccatcttcttcaaggacgacggcaactacaagacccgcgccgaggtgaagttcgagggcgacaccctggtgaaccgcatcgagctgaagggcatcgacttcaaggaggacggcaacatcctggggcacaagctggagtacaactacaacagccacaacgtctatatcatggccgacaagcagaagaacggcatcaaggtgaacttcaagatccgccacaacatcgaggacggcagcgtgcagctcgccgaccactaccagcagaacacccccatcggcgacggccccgtgctgctgcccgacaaccactacctgagcacccagtccaagctgagcaaagaccccaacgagaagcgcgatcacatggtcctgctggagttcgtgaccgccgccgggatcactctcggcatggacgagctgtacaagtaaagcggccgcgactctagagtcgacctgcaggcatgcaagcttgatatcaagcttatcgataatcaacctctggattacaaaatttgtgaaagattgactggtattcttaactatgttgctccttttacgctatgtggatacgctgctttaatgcctttgtatcatgctattgcttcccgtatggctttcattttctcctccttgtataaatcctggttgctgtctctttatgaggagttgtggcccgttgtcaggcaacgtggcgtggtgtgcactgtgtttgctgacgcaacccccactggttggggcattgccaccacctgtcagctcctttccgggactttcgctttccccctccctattgccacggcggaactcatcgccgcctgccttgcccgctgctggacaggggctcggctgttgggcactgacaattccgtggtgttgtcggggaaatcatcgtcctttccttggctgctcgcctgtgttgccacctggattctgcgcgggacgtccttctgctacgtcccttcggccctcaatccagcggaccttccttcccgcggcctgctgccggctctgcggcctcttccgcgtcttcgccttcgccctcagacgagtcggatctccctttgggccgcctccccgcat

SEQ ID NO: 8 - RNA, 573 nt, Homo sapiens
ctgggggttctatttgggaaggtattcagccaaacgaccatctgccgctttgaggctctgcagcttagcttcaagaacatgtgtaagctgcggcccttgctgcagaagtgggtggaggaagctgacaacaatgaaaatcttcaggagatatgcaaagcagaaaccctcgtgcaggcccgaaagagaaagcgaaccagtatcgagaaccgagtgagaggcaacctggagaatttgttcctgcagtgcccgaaacccacactgcagcagatcagccacatcgcccagcagcttgggctcgagaaggatgtggtccgagtgtggttctgtaaccggcgccagaagggcaagcgatcaagcagcgactatgcacaacgagaggattttgaggctgctgggtctcctttctcagggggaccagtgtcctttcctctggccccagggccccattttggtaccccaggctatgggagccctcacttcactgcactgtactcctcggtccctttccctgagggggaagcctttccccctgtctccgtcaccactctgggctctcccatgcattcaaactga

SEQ ID NO: 9 - RNA, 954 nt, Homo sapiens
atgtacaacatgatggagacggagctgaagccgccgggcccgcagcaaacttcggggggcggcggcggcaactccaccgcggcggcggccggcggcaaccagaaaaacagcccggaccgcgtcaagcggcccatgaatgccttcatggtgtggtcccgcgggcagcggcgcaagatggcccaggagaaccccaagatgcacaactcggagatcagcaagcgcctgggcgccgagtggaaacttttgtcggagacggagaagcggccgttcatcgacgaggctaagcggctgcgagcgctgcacatgaaggagcacccggattataaataccggccccggcggaaaaccaagacgctcatgaagaaggataagtacacgctgcccggcgggctgctggcccccggcggcaatagcatggcgagcggggtcggggtgggcgccggcctgggcgcgggcgtgaaccagcgcatggacagttacgcgcacatgaacggctggagcaacggcagctacagcatgatgcaggaccagctgggctacccgcagcacccgggcctcaatgcgcacggcgcagcgcagatgcagcccatgcaccgctacgacgtgagcgccctgcagtacaactccatgaccagctcgcagacctacatgaacggctcgcccacctacagcatgtcctactcgcagcagggcacccctggcatggctcttggctccatgggttcggtggtcaagtccgaggccagctccagcccccctgtggttacctcttcctcccactccagggcgccctgccaggccggggacctccgggacatgatcagcatgtatctccccggcgccgaggtgccggaacccgccgcccccagcagacttcacatgtcccagcactaccagagcggcccggtgcccggcacggccattaacggcacactgcccctctcacacatgtga

SEQ ID NO: 10 - RNA, 1365 nt, Homo sapiens
ctggatttttttcgggtagtggaaaaccagcagcctcccgcgacgatgcccctcaacgttagcttcaccaacaggaactatgacctcgactacgactcggtgcagccgtatttctactgcgacgaggaggagaacttctaccagcagcagcagcagagcgagctgcagcccccggcgcccagcgaggatatctggaagaaattcgagctgctgcccaccccgcccctgtcccctagccgccgctccgggctctgctcgccctcctacgttgcggtcacacccttctcccttcggggagacaacgacggcggtggcgggagcttctccacggccgaccagctggagatggtgaccgagctgctgggaggagacatggtgaaccagagtttcatctgcgacccggacgacgagaccttcatcaaaaacatcatcatccaggactgtatgtggagcggcttctcggccgccgccaagctcgtctcagagaagctggcctcctaccaggctgcgcgcaaagacagcggcagcccgaaccccgcccgcggccacagcgtctgctccacctccagcttgtacctgcaggatctgagcgccgccgcctcagagtgcatcgacccctcggtggtcttcccctaccctctcaacgacagcagctcgcccaagtcctgcgcctcgcaagactccagcgccttctctccgtcctcggattctctgctctcctcgacggagtcctccccgcagggcagccccgagcccctggtgctccatgaggagacaccgcccaccaccagcagcgactctgaggaggaacaagaagatgaggaagaaatcgatgttgtttctgtggaaaagaggcaggctcctggcaaaaggtcagagtctggatcaccttctgctggaggccacagcaaacctcctcacagcccactggtcctcaagaggtgccacgtctccacacatcagcacaactacgcagcgcctccctccactcggaaggactatcctgctgccaagagggtcaagttggacagtgtcagagtcctgagacagatcagcaacaaccgaaaatgcaccagccccaggtcctcggacaccgaggagaatgtcaagaggcgaacacacaacgtcttggagcgccagaggaggaacgagctaaaacggagcttttttgccctgcgtgaccagatcccggagttggaaaacaatgaaaaggcccccaaggtagttatccttaaaaaagccacagcatacatcctgtccgtccaagcagaggagcaaaagctcatttctgaagaggacttgttgcggaaacgacgagaacagttgaaacacaaacttgaacagctacggaactcttgtgcgtaa

SEQ ID NO: 11 - RNA, 1542 nt, Homo sapiens
atgaggcagccacctggcgagtctgacatggctgtcagcgacgcgctgctcccatctttctccacgttcgcgtctggcccggcgggaagggagaagacactgcgtcaagcaggtgccccgaataaccgctggcgggaggagctctcccacatgaagcgacttcccccagtgcttcccggccgcccctatgacctggcggcggcgaccgtggccacagacctggagagcggcggagccggtgcggcttgcggcggtagcaacctggcgcccctacctcggagagagaccgaggagttcaacgatctcctggacctggactttattctctccaattcgctgacccatcctccggagtcagtggccgccaccgtgtcctcgtcagcgtcagcctcctcttcgtcgtcgccgtcgagcagcggccctgccagcgcgccctccacctgcagcttcacctatccgatccgggccgggaacgacccgggcgtggcgccgggcggcacgggcggaggcctcctctatggcagggagtccgctccccctccgacggctcccttcaacctggcggacatcaacgacgtgagcccctcgggcggcttcgtggccgagctcctgcggccagaattggacccggtgtacattccgccgcagcagccgcagccgccaggtggcgggctgatgggcaagttcgtgctgaaggcgtcgctgagcgcccctggcagcgagtacggcagcccgtcggtcatcagcgtcagcaaaggcagccctgacggcagccacccggtggtggtggcgccctacaacggcgggccgccgcgcacgtgccccaagatcaagcaggaggcggtctcttcgtgcacccacttgggcgctggaccccctctcagcaatggccaccggccggctgcacacgacttccccctggggcggcagctccccagcaggactaccccgaccctgggtcttgaggaagtgctgagcagcagggactgtcaccctgccctgccgcttcctcccggcttccatccccacccggggcccaattacccatccttcctgcccgatcagatgcagccgcaagtcccgccgctccattaccaaggtcagtcccggggatttgtagctcgggctggggagccctgtgtgtgctggccccacttcgggacacacgggatgatgctcaccccaccttcttcacccctagagctcatgccacccggttcctgcatgccagaggagcccaagccaaagaggggaagacgatcgtggccccggaaaaggaccgccacccacacttgtgattacgcgggctgcggcaaaacctacacaaagagttcccatctcaaggcacacctgcgaacccacacaggtgagaaaccttaccactgtgactgggacggctgtggatggaaattcgcccgctcagatgaactgaccaggcactaccgtaaacacacggggcaccgcccgttccagtgccaaaaatgcgaccgagcattttccaggtcggaccacctcgccttacacatgaagaggcatttttaa

SEQ ID NO: 12 - RNA, 1017 nt, Homo sapiens
atggtggtcatggcgccccgaaccctcttcctgctgctctcgggggccctgaccctgaccgagacctgggcgggctcccactccatgaggtatttcagcgccgccgtgtcccggcccggccgcggggagccccgcttcatcgccatgggctacgtggacgacacgcagttcgtgcggttcgacagcgactcggcgtgtccgaggatggagccgcgggcgccgtgggtggagcaggaggggccggagtattgggaagaggagacacggaacaccaaggcccacgcacagactgacagaatgaacctgcagaccctgcgcggctactacaaccagagcgaggccagttctcacaccctccagtggatgattggctgcgacctggggtccgacggacgcctcctccgcgggtatgaacagtatgcctacgatggcaaggattacctcgccctgaacgaggacctgcgctcctggaccgcagcggacactgcggctcagatctccaagcgcaagtgtgaggcggccaatgtggctgaacaaaggagagcctacctggagggcacgtgcgtggagtggctccacagatacctggagaacgggaaggagatgctgcagcgcgcggacccccccaagacacacgtgacccaccaccctgtctttgactatgaggccaccctgaggtgctgggccctgggcttctaccctgcggagatcatactgacctggcagcgggatggggaggaccagacccaggacgtggagctcgtggagaccaggcctgcaggggatggaaccttccagaagtgggcagctgtggtggtgccttctggagaggagcagagatacacgtgccatgtgcagcatgaggggctgccggagcccctcatgctgagatggaagcagtcttccctgcccaccatccccatcatgggtatcgttgctggcctggttgtccttgcagctgtagtcactggagctgcggtcgctgctgtgctgtggagaaagaagagctcagattga

SEQ ID NO: 13 - RNA, 1002 nt, Homo sapiens
atggggcccctcccagccccttcctgcacacagcgcatcacctggaaggggctcctgctcacagcatcacttttaaacttctggaacccgcccaccactgccgaagtcacgattgaagcccagccacccaaagtttctgaggggaaggatgttcttctacttgtccacaatttgccccagaatcttcctggctacttctggtacaaaggggaaatgacggacctctaccattacattatatcgtatatagttgatggtaaaataattatatatgggcctgcatacagtggaagagaaacagtatattccaacgcatccctgctgatccagaatgtcacccggaaggatgcaggaacctacaccttacacatcataaagcgaggtgatgagactagagaagaaattcgacatttcaccttcaccttatactcgaagctgcccatcccctacatcaccatcaacaacttaaaccccagggagaataaggatgtcttagccttcacctgtgaacctaagagtgagaactacacctacatttggtggctaaacggtcagagcctccccgtcagtcccggggtaaagcgacccattgaaaacaggatactcattctacccagtgtcacgagaaatgaaacaggaccctatcaatgtgaaatacgggaccgatatggtggcctccgcagtaacccagtcatcctaaatgtcctctatggtccagacctccccagaatttacccttcattcacctattaccgttcaggagaaaacctcgacttgtcctgcttcacggaatctaacccaccggcagagtatttttggacaattaatgggaagtttcagcaatcaggacaaaagctctttatcccccaaattactagaaatcatagcgggctctatgcttgctctgttcataactcagccactggcaaggaaatctccaaatccatgacagtcaaagtctctggtccctgccatggagacctgacagagtctcagtcatga